European Patent Application EP 4 169 950 A1, published April 26, 2023. Title: ANTI-LILRB1 ANTIBODY AND USES THEREOF. Applicant: LG CHEM, LTD. The sequence listing filed with the application follows.

SEQUENCE LISTING (230 sequences)

SEQ ID NO: 1 - protein, 11 aa, Artificial Sequence
  Synthetic (5_CDR-L1)
RASQSIANYLN

SEQ ID NO: 2 - protein, 7 aa, Artificial Sequence
  Synthetic (5_CDR-L2)
ATSTLQS

SEQ ID NO: 3 - protein, 9 aa, Artificial Sequence
  Synthetic (5_CDR-L3)
QQSYSFPWT

SEQ ID NO: 4 - protein, 5 aa, Artificial Sequence
  Synthetic (5_CDR-H1)
AYGIH

SEQ ID NO: 5 - protein, 17 aa, Artificial Sequence
  Synthetic (5_CDR-H2)
WIIPLSGGAHYAQKFQG

SEQ ID NO: 6 - protein, 10 aa, Artificial Sequence
  Synthetic (5_CDR-H3)
LYGWAEYFDV

SEQ ID NO: 7 - protein, 107 aa, Artificial Sequence
  Synthetic (5_LightChain_VariableRegion)
DIQMTQSPSSLSASVGDRVTITCRASQSIANYLNWYQQKPGKAPKLLIYATSTLQSGVPSRFSGSGSGTDFTLTISSLQPEDFATYYCQQSYSFPWTFGQGTKVEIK

SEQ ID NO: 8 - DNA, 321 bp, Artificial Sequence
  Synthetic (5_LightChain_VariableRegion_gene)
gacattcaaatgacgcagagtccctcctcactgagtgctagcgtgggcgatcgtgtgacaattacttgtcgcgctagccagtctatcgcaaattacctgaactggtatcagcagaaaccgggcaaggcgccaaaattgctgatttacgcaacttccactctgcagtctggtgtaccgtcccgtttctctggcagcggttctggtacggattttaccctgaccatctcaagcctccagcctgaagattttgccacctattattgtcagcaatcttactcttttccgtggacgttcgggcagggaactaaagtggaaattaaa

SEQ ID NO: 9 - protein, 119 aa, Artificial Sequence
  Synthetic (5_HeavyChain_VariableRegion)
QVQLVQSGAEVKKPGSSVKVSCKASGGTFSAYGIHWVRQAPGQGLEWMGWIIPLSGGAHYAQKFQGRVTITADESTSTAYMELSSLRSEDTAVYYCARLYGWAEYFDVWGQGTLVTVSS

SEQ ID NO: 10 - DNA, 357 bp, Artificial Sequence
  Synthetic (5_HeavyChain_VariableRegion_gene)
caagttcagctggtccagagcggcgcagaggtgaagaagcccggcagttctgttaaggtttcctgcaaagcctcaggcgggacttttagtgcatacggtatccattgggtgcggcaggcgcccggccagggtctcgaatggatggggtggattatcccactgtctggtggtgcacattatgcacaaaaattccaaggccgcgtaactattaccgccgacgaatcaacctccaccgcctacatggaactcagctctctgaggtcagaagacacggccgtctattattgcgccagactgtacggttgggcagaatacttcgatgtttggggtcagggtactctggttaccgtctcatcg

SEQ ID NO: 11 - protein, 214 aa, Artificial Sequence
  Synthetic (5_LightChain_Kappa)
DIQMTQSPSSLSASVGDRVTITCRASQSIANYLNWYQQKPGKAPKLLIYATSTLQSGVPSRFSGSGSGTDFTLTISSLQPEDFATYYCQQSYSFPWTFGQGTKVEIKRTVAAPSVFIFPPSDEQLKSGTASVVCLLNNFYPREAKVQWKVDNALQSGNSQESVTEQDSKDSTYSLSSTLTLSKADYEKHKVYACEVTHQGLSSPVTKSFNRGEC

SEQ ID NO: 12 - protein, 445 aa, Artificial Sequence
  Synthetic (5_HeavyChain)
QVQLVQSGAEVKKPGSSVKVSCKASGGTFSAYGIHWVRQAPGQGLEWMGWIIPLSGGAHYAQKFQGRVTITADESTSTAYMELSSLRSEDTAVYYCARLYGWAEYFDVWGQGTLVTVSSASTKGPSVFPLAPCSRSTSESTAALGCLVKDYFPEPVTVSWNSGALTSGVHTFPAVLQSSGLYSLSSVVTVPSSSLGTKTYTCNVDHKPSNTKVDKRVESKYGPPCPPCPAPEAAGGPSVFLFPPKPKDTLMISRTPEVTCVVVDVSQEDPEVQFNWYVDGVEVHNAKTKPREEQFNSTYRVVSVLTVLHQDWLNGKEYKCKVSNKGLPSSIEKTISKAKGQPREPQVYTLPPSQEEMTKNQVSLTCLVKGFYPSDIAVEWESNGQPENNYKTTPPVLDSDGSFFLYSRLTVDKSRWQEGNVFSCSVMHEALHNHYTQKSLSLSLG

SEQ ID NO: 13 - protein, 11 aa, Artificial Sequence
  Synthetic (6_CDR-L1)
RASQSISNYLN

SEQ ID NO: 14 - protein, 7 aa, Artificial Sequence
  Synthetic (6_CDR-L2)
AASTLQS

SEQ ID NO: 15 - protein, 9 aa, Artificial Sequence
  Synthetic (6_CDR-L3)
QQSYSFPWT

SEQ ID NO: 16 - protein, 5 aa, Artificial Sequence
  Synthetic (6_CDR-H1)
SYTIS

SEQ ID NO: 17 - protein, 17 aa, Artificial Sequence
  Synthetic (6_CDR-H2)
WISPELGTSNYAQKFQG

SEQ ID NO: 18 - protein, 12 aa, Artificial Sequence
  Synthetic (6_CDR-H3)
LRYGQTLYGFDI

SEQ ID NO: 19 - protein, 107 aa, Artificial Sequence
  Synthetic (6_LightChain_VariableRegion)
DIQMTQSPSSLSASVGDRVTITCRASQSISNYLNWYQQKPGKAPKLLIYAASTLQSGVPSRFSGSGSGTDFTLTISSLQPEDFATYYCQQSYSFPWTFGQGTKVEIK

SEQ ID NO: 20 - DNA, 321 bp, Artificial Sequence
  Synthetic (6_LightChain_VariableRegion_gene)
gacattcaaatgacgcagagtccctcctcactgagtgctagcgtgggcgatcgtgtgacaattacttgtcgcgctagccagtctatctctaattacctgaactggtatcagcagaaaccgggcaaggcgccaaaattgctgatttacgcagcatccactctgcagtctggtgtaccgtcccgtttctctggcagcggttctggtacggattttaccctgaccatctcaagcctccagcctgaagattttgccacctattattgtcagcaatcttactcttttccgtggacgttcgggcagggaactaaagtggaaattaaa

SEQ ID NO: 21 - protein, 121 aa, Artificial Sequence
  Synthetic (6_HeavyChain_VariableRegion)
QVQLVQSGAEVKKPGSSVKVSCKASGGTFSSYTISWVRQAPGQGLEWMGWISPELGTSNYAQKFQGRVTITADESTSTAYMELSSLRSEDTAVYYCARLRYGQTLYGFDIWGQGTLVTVSS

SEQ ID NO: 22 - DNA, 363 bp, Artificial Sequence
  Synthetic (6_HeavyChain_VariableRegion_gene)
caagttcagctggtccagagcggcgcagaggtgaagaagcccggcagttctgttaaggtttcctgcaaagcctcaggcgggacttttagttcttacaccatttcttgggtgcggcaggcgcccggccagggtctcgaatggatggggtggatttctccagaactgggtacctctaactatgcacaaaaattccaaggccgcgtaactattaccgccgacgaatcaacctccaccgcctacatggaactcagctctctgaggtcagaagacacggccgtctattattgcgccagactgcgttacggtcagactctgtacggtttcgatatctggggtcagggtactctggttaccgtctcatcg

SEQ ID NO: 23 - protein, 214 aa, Artificial Sequence
  Synthetic (6_LightChain_Kappa)
DIQMTQSPSSLSASVGDRVTITCRASQSISNYLNWYQQKPGKAPKLLIYAASTLQSGVPSRFSGSGSGTDFTLTISSLQPEDFATYYCQQSYSFPWTFGQGTKVEIKRTVAAPSVFIFPPSDEQLKSGTASVVCLLNNFYPREAKVQWKVDNALQSGNSQESVTEQDSKDSTYSLSSTLTLSKADYEKHKVYACEVTHQGLSSPVTKSFNRGEC

SEQ ID NO: 24 - protein, 447 aa, Artificial Sequence
  Synthetic (6_HeavyChain)
QVQLVQSGAEVKKPGSSVKVSCKASGGTFSSYTISWVRQAPGQGLEWMGWISPELGTSNYAQKFQGRVTITADESTSTAYMELSSLRSEDTAVYYCARLRYGQTLYGFDIWGQGTLVTVSSASTKGPSVFPLAPCSRSTSESTAALGCLVKDYFPEPVTVSWNSGALTSGVHTFPAVLQSSGLYSLSSVVTVPSSSLGTKTYTCNVDHKPSNTKVDKRVESKYGPPCPPCPAPEAAGGPSVFLFPPKPKDTLMISRTPEVTCVVVDVSQEDPEVQFNWYVDGVEVHNAKTKPREEQFNSTYRVVSVLTVLHQDWLNGKEYKCKVSNKGLPSSIEKTISKAKGQPREPQVYTLPPSQEEMTKNQVSLTCLVKGFYPSDIAVEWESNGQPENNYKTTPPVLDSDGSFFLYSRLTVDKSRWQEGNVFSCSVMHEALHNHYTQKSLSLSLG

SEQ ID NO: 25 - protein, 11 aa, Artificial Sequence
  Synthetic (7_CDR-L1)
RASQSISNWLN

SEQ ID NO: 26 - protein, 7 aa, Artificial Sequence
  Synthetic (7_CDR-L2)
GTSSLQS

SEQ ID NO: 27 - protein, 9 aa, Artificial Sequence
  Synthetic (7_CDR-L3)
QQSYSFPFT

SEQ ID NO: 28 - protein, 5 aa, Artificial Sequence
  Synthetic (7_CDR-H1)
SYGMH

SEQ ID NO: 29 - protein, 17 aa, Artificial Sequence
  Synthetic (7_CDR-H2)
WIIPVSGGATYAQKFQG

SEQ ID NO: 30 - protein, 11 aa, Artificial Sequence
  Synthetic (7_CDR-H3)
GSWAYYAEFDY

SEQ ID NO: 31 - protein, 107 aa, Artificial Sequence
  Synthetic (7_LightChain_VariableRegion)
DIQMTQSPSSLSASVGDRVTITCRASQSISNWLNWYQQKPGKAPKLLIYGTSSLQSGVPSRFSGSGSGTDFTLTISSLQPEDFATYYCQQSYSFPFTFGQGTKVEIK

SEQ ID NO: 32 - DNA, 321 bp, Artificial Sequence
  Synthetic (7_LightChain_VariableRegion_gene)
gacattcaaatgacgcagagtccctcctcactgagtgctagcgtgggcgatcgtgtgacaattacttgtcgcgctagccagtctatctctaattggctgaactggtatcagcagaaaccgggcaaggcgccaaaattgctgatttacggtacttcctctctgcagtctggtgtaccgtcccgtttctctggcagcggttctggtacggattttaccctgaccatctcaagcctccagcctgaagattttgccacctattattgtcagcaatcttactcttttccgtttacgttcgggcagggaactaaagtggaaattaaa

SEQ ID NO: 33 - protein, 120 aa, Artificial Sequence
  Synthetic (7_HeavyChain_VariableRegion)
QVQLVQSGAEVKKPGSSVKVSCKASGGTFSSYGMHWVRQAPGQGLEWMGWIIPVSGGATYAQKFQGRVTITADESTSTAYMELSSLRSEDTAVYYCARGSWAYYAEFDYWGQGTLVTVSS

SEQ ID NO: 34 - DNA, 360 bp, Artificial Sequence
  Synthetic (7_HeavyChain_VariableRegion_gene)
caagttcagctggtccagagcggcgcagaggtgaagaagcccggcagttctgttaaggtttcctgcaaagcctcaggcgggacttttagttcttacggtatgcattgggtgcggcaggcgcccggccagggtctcgaatggatggggtggattatcccagtttctggtggtgcaacctatgcacaaaaattccaaggccgcgtaactattaccgccgacgaatcaacctccaccgcctacatggaactcagctctctgaggtcagaagacacggccgtctattattgcgccagaggttcttgggcatactacgctgaattcgattactggggtcagggcactttagtgaccgtctcatcg

SEQ ID NO: 35 - protein, 214 aa, Artificial Sequence
  Synthetic (7_LightChain_Kappa)
DIQMTQSPSSLSASVGDRVTITCRASQSISNWLNWYQQKPGKAPKLLIYGTSSLQSGVPSRFSGSGSGTDFTLTISSLQPEDFATYYCQQSYSFPFTFGQGTKVEIKRTVAAPSVFIFPPSDEQLKSGTASVVCLLNNFYPREAKVQWKVDNALQSGNSQESVTEQDSKDSTYSLSSTLTLSKADYEKHKVYACEVTHQGLSSPVTKSFNRGEC

SEQ ID NO: 36 - protein, 446 aa, Artificial Sequence
  Synthetic (7_HeavyChain)
QVQLVQSGAEVKKPGSSVKVSCKASGGTFSSYGMHWVRQAPGQGLEWMGWIIPVSGGATYAQKFQGRVTITADESTSTAYMELSSLRSEDTAVYYCARGSWAYYAEFDYWGQGTLVTVSSASTKGPSVFPLAPCSRSTSESTAALGCLVKDYFPEPVTVSWNSGALTSGVHTFPAVLQSSGLYSLSSVVTVPSSSLGTKTYTCNVDHKPSNTKVDKRVESKYGPPCPPCPAPEAAGGPSVFLFPPKPKDTLMISRTPEVTCVVVDVSQEDPEVQFNWYVDGVEVHNAKTKPREEQFNSTYRVVSVLTVLHQDWLNGKEYKCKVSNKGLPSSIEKTISKAKGQPREPQVYTLPPSQEEMTKNQVSLTCLVKGFYPSDIAVEWESNGQPENNYKTTPPVLDSDGSFFLYSRLTVDKSRWQEGNVFSCSVMHEALHNHYTQKSLSLSLG

SEQ ID NO: 37 - protein, 11 aa, Artificial Sequence
  Synthetic (8_CDR-L1)
RASQSISSYLN

SEQ ID NO: 38 - protein, 7 aa, Artificial Sequence
  Synthetic (8_CDR-L2)
AASTLQS

SEQ ID NO: 39 - protein, 9 aa, Artificial Sequence
  Synthetic (8_CDR-L3)
QQSYSFPYT

SEQ ID NO: 40 - protein, 5 aa, Artificial Sequence
  Synthetic (8_CDR-H1)
SYGIH

SEQ ID NO: 41 - protein, 17 aa, Artificial Sequence
  Synthetic (8_CDR-H2)
WIIPISGTTNYAQKFQG

SEQ ID NO: 42 - protein, 11 aa, Artificial Sequence
  Synthetic (8_CDR-H3)
VGGVGLYVFDV

SEQ ID NO: 43 - protein, 107 aa, Artificial Sequence
  Synthetic (8_LightChain_VariableRegion)
DIQMTQSPSSLSASVGDRVTITCRASQSISSYLNWYQQKPGKAPKLLIYAASTLQSGVPSRFSGSGSGTDFTLTISSLQPEDFATYYCQQSYSFPYTFGQGTKVEIK

SEQ ID NO: 44 - DNA, 321 bp, Artificial Sequence
  Synthetic (8_LightChain_VariableRegion_gene)
gacattcaaatgacgcagagtccctcctcactgagtgctagcgtgggcgatcgtgtgacaattacttgtcgcgctagccagtctatctcttcttacctgaactggtatcagcagaaaccgggcaaggcgccaaaattgctgatttacgcagcatccactctgcagtctggtgtaccgtcccgtttctctggcagcggttctggtacggattttaccctgaccatctcaagcctccagcctgaagattttgccacctattattgtcagcaatcttactcttttccgtacacgttcgggcagggaactaaagtggaaattaaa

SEQ ID NO: 45 - protein, 120 aa, Artificial Sequence
  Synthetic (8_HeavyChain_VariableRegion)
QVQLVQSGAEVKKPGSSVKVSCKASGGTFSSYGIHWVRQAPGQGLEWMGWIIPISGTTNYAQKFQGRVTITADESTSTAYMELSSLRSEDTAVYYCARVGGVGLYVFDVWGQGTLVTVSS

SEQ ID NO: 46 - DNA, 360 bp, Artificial Sequence
  Synthetic (8_HeavyChain_VariableRegion_gene)
caagttcagctggtccagagcggcgcagaggtgaagaagcccggcagttctgttaaggtttcctgcaaagcctcaggcgggacttttagttcttacggtatccattgggtgcggcaggcgcccggccagggtctcgaatggatggggtggattatcccaatctctggtaccaccaactatgcacaaaaattccaaggccgcgtaactattaccgccgacgaatcaacctccaccgcctacatggaactcagctctctgaggtcagaagacacggccgtctattattgcgccagagttggtggtgttggtctgtacgttttcgatgtttggggtcagggtactctggttaccgtctcatcg

SEQ ID NO: 47 - protein, 214 aa, Artificial Sequence
  Synthetic (8_LightChain_Kappa)
DIQMTQSPSSLSASVGDRVTITCRASQSISSYLNWYQQKPGKAPKLLIYAASTLQSGVPSRFSGSGSGTDFTLTISSLQPEDFATYYCQQSYSFPYTFGQGTKVEIKRTVAAPSVFIFPPSDEQLKSGTASVVCLLNNFYPREAKVQWKVDNALQSGNSQESVTEQDSKDSTYSLSSTLTLSKADYEKHKVYACEVTHQGLSSPVTKSFNRGEC

SEQ ID NO: 48 - protein, 446 aa, Artificial Sequence
  Synthetic (8_HeavyChain)
QVQLVQSGAEVKKPGSSVKVSCKASGGTFSSYGIHWVRQAPGQGLEWMGWIIPISGTTNYAQKFQGRVTITADESTSTAYMELSSLRSEDTAVYYCARVGGVGLYVFDVWGQGTLVTVSSASTKGPSVFPLAPCSRSTSESTAALGCLVKDYFPEPVTVSWNSGALTSGVHTFPAVLQSSGLYSLSSVVTVPSSSLGTKTYTCNVDHKPSNTKVDKRVESKYGPPCPPCPAPEAAGGPSVFLFPPKPKDTLMISRTPEVTCVVVDVSQEDPEVQFNWYVDGVEVHNAKTKPREEQFNSTYRVVSVLTVLHQDWLNGKEYKCKVSNKGLPSSIEKTISKAKGQPREPQVYTLPPSQEEMTKNQVSLTCLVKGFYPSDIAVEWESNGQPENNYKTTPPVLDSDGSFFLYSRLTVDKSRWQEGNVFSCSVMHEALHNHYTQKSLSLSLG

SEQ ID NO: 49 - protein, 11 aa, Artificial Sequence
  Synthetic (9_CDR-L1)
RASQSISNYLN

SEQ ID NO: 50 - protein, 7 aa, Artificial Sequence
  Synthetic (9_CDR-L2)
AASSLQS

SEQ ID NO: 51 - protein, 9 aa, Artificial Sequence
  Synthetic (9_CDR-L3)
QQSYSFPWT

SEQ ID NO: 52 - protein, 5 aa, Artificial Sequence
  Synthetic (9_CDR-H1)
SYAIH

SEQ ID NO: 53 - protein, 17 aa, Artificial Sequence
  Synthetic (9_CDR-H2)
WIVPGLGVTNYAQKFQG

SEQ ID NO: 54 - protein, 12 aa, Artificial Sequence
  Synthetic (9_CDR-H3)
QATLYQTEYMDV

SEQ ID NO: 55 - protein, 107 aa, Artificial Sequence
  Synthetic (9_LightChain_VariableRegion)
DIQMTQSPSSLSASVGDRVTITCRASQSISNYLNWYQQKPGKAPKLLIYAASSLQSGVPSRFSGSGSGTDFTLTISSLQPEDFATYYCQQSYSFPWTFGQGTKVEIK

SEQ ID NO: 56 - DNA, 321 bp, Artificial Sequence
  Synthetic (9_LightChain_VariableRegion_gene)
gacattcaaatgacgcagagtccctcctcactgagtgctagcgtgggcgatcgtgtgacaattacttgtcgcgctagccagtctatctctaattacctgaactggtatcagcagaaaccgggcaaggcgccaaaattgctgatttacgcagcatcctctctgcagtctggtgtaccgtcccgtttctctggcagcggttctggtacggattttaccctgaccatctcaagcctccagcctgaagattttgccacctattattgtcagcaatcttactcttttccgtggacgttcgggcagggaactaaagtggaaattaaa

SEQ ID NO: 57 - protein, 121 aa, Artificial Sequence
  Synthetic (9_HeavyChain_VariableRegion)
QVQLVQSGAEVKKPGSSVKVSCKASGGTFSSYAIHWVRQAPGQGLEWMGWIVPGLGVTNYAQKFQGRVTITADESTSTAYMELSSLRSEDTAVYYCARQATLYQTEYMDVWGQGTLVTVSS

SEQ ID NO: 58 - DNA, 363 bp, Artificial Sequence
  Synthetic (9_HeavyChain_VariableRegion_gene)
caagttcagctggtccagagcggcgcagaggtgaagaagcccggcagttctgttaaggtttcctgcaaagcctcaggcgggacttttagttcttacgcaatccattgggtgcggcaggcgcccggccagggtctcgaatggatggggtggattgttccaggtctgggtgttaccaactatgcacaaaaattccaaggccgcgtaactattaccgccgacgaatcaacctccaccgcctacatggaactcagctctctgaggtcagaagacacggccgtctattattgcgccagacaggcaactctgtaccagactgaatacatggatgtttggggtcagggtactctggttaccgtctcatcg

SEQ ID NO: 59 - protein, 214 aa, Artificial Sequence
  Synthetic (9_LightChain_Kappa)
DIQMTQSPSSLSASVGDRVTITCRASQSISNYLNWYQQKPGKAPKLLIYAASSLQSGVPSRFSGSGSGTDFTLTISSLQPEDFATYYCQQSYSFPWTFGQGTKVEIKRTVAAPSVFIFPPSDEQLKSGTASVVCLLNNFYPREAKVQWKVDNALQSGNSQESVTEQDSKDSTYSLSSTLTLSKADYEKHKVYACEVTHQGLSSPVTKSFNRGEC

SEQ ID NO: 60 - protein, 447 aa, Artificial Sequence
  Synthetic (9_HeavyChain)
QVQLVQSGAEVKKPGSSVKVSCKASGGTFSSYAIHWVRQAPGQGLEWMGWIVPGLGVTNYAQKFQGRVTITADESTSTAYMELSSLRSEDTAVYYCARQATLYQTEYMDVWGQGTLVTVSSASTKGPSVFPLAPCSRSTSESTAALGCLVKDYFPEPVTVSWNSGALTSGVHTFPAVLQSSGLYSLSSVVTVPSSSLGTKTYTCNVDHKPSNTKVDKRVESKYGPPCPPCPAPEAAGGPSVFLFPPKPKDTLMISRTPEVTCVVVDVSQEDPEVQFNWYVDGVEVHNAKTKPREEQFNSTYRVVSVLTVLHQDWLNGKEYKCKVSNKGLPSSIEKTISKAKGQPREPQVYTLPPSQEEMTKNQVSLTCLVKGFYPSDIAVEWESNGQPENNYKTTPPVLDSDGSFFLYSRLTVDKSRWQEGNVFSCSVMHEALHNHYTQKSLSLSLG

SEQ ID NO: 61 - protein, 11 aa, Artificial Sequence
  Synthetic (10_CDR-L1)
RASQSISNYLN

SEQ ID NO: 62 - protein, 7 aa, Artificial Sequence
  Synthetic (10_CDR-L2)
AASNLQS

SEQ ID NO: 63 - protein, 9 aa, Artificial Sequence
  Synthetic (10_CDR-L3)
QQSYSFPFT

SEQ ID NO: 64 - protein, 5 aa, Artificial Sequence
  Synthetic (10_CDR-H1)
SHYMH

SEQ ID NO: 65 - protein, 17 aa, Artificial Sequence
  Synthetic (10_CDR-H2)
WISPYLGSTNYAQKFQG

SEQ ID NO: 66 - protein, 12 aa, Artificial Sequence
  Synthetic (10_CDR-H3)
DETGSTYGAFDY

SEQ ID NO: 67 - protein, 107 aa, Artificial Sequence
  Synthetic (10_LightChain_VariableRegion)
DIQMTQSPSSLSASVGDRVTITCRASQSISNYLNWYQQKPGKAPKLLIYAASNLQSGVPSRFSGSGSGTDFTLTISSLQPEDFATYYCQQSYSFPFTFGQGTKVEIK

SEQ ID NO: 68 - DNA, 321 bp, Artificial Sequence
  Synthetic (10_LightChain_VariableRegion_gene)
gacattcaaatgacgcagagtccctcctcactgagtgctagcgtgggcgatcgtgtgacaattacttgtcgcgctagccagtctatctctaattacctgaactggtatcagcagaaaccgggcaaggcgccaaaattgctgatttacgcagcatccaatctgcagtctggtgtaccgtcccgtttctctggcagcggttctggtacggattttaccctgaccatctcaagcctccagcctgaagattttgccacctattattgtcagcaatcttactcttttccgtttacgttcgggcagggaactaaagtggaaattaaa

SEQ ID NO: 69 - protein, 121 aa, Artificial Sequence
  Synthetic (10_HeavyChain_VariableRegion)
QVQLVQSGAEVKKPGSSVKVSCKASGGTFSSHYMHWVRQAPGQGLEWMGWISPYLGSTNYAQKFQGRVTITADESTSTAYMELSSLRSEDTAVYYCARDETGSTYGAFDYWGQGTLVTVSS

SEQ ID NO: 70 - DNA, 363 bp, Artificial Sequence
  Synthetic (10_HeavyChain_VariableRegion_gene)
caagttcagctggtccagagcggcgcagaggtgaagaagcccggcagttctgttaaggtttcctgcaaagcctcaggcgggacttttagttctcattacatgcattgggtgcggcaggcgcccggccagggtctcgaatggatggggtggatttctccatacctgggttctaccaactatgcacaaaaattccaaggccgcgtaactattaccgccgacgaatcaacctccaccgcctacatggaactcagctctctgaggtcagaagacacggccgtctattattgcgccagagatgaaactggttctacttacggtgcattcgattactggggtcagggtactctggttaccgtctcatcg

SEQ ID NO: 71 - protein, 214 aa, Artificial Sequence
  Synthetic (10_LightChain_Kappa)
DIQMTQSPSSLSASVGDRVTITCRASQSISNYLNWYQQKPGKAPKLLIYAASNLQSGVPSRFSGSGSGTDFTLTISSLQPEDFATYYCQQSYSFPFTFGQGTKVEIKRTVAAPSVFIFPPSDEQLKSGTASVVCLLNNFYPREAKVQWKVDNALQSGNSQESVTEQDSKDSTYSLSSTLTLSKADYEKHKVYACEVTHQGLSSPVTKSFNRGEC

SEQ ID NO: 72 - protein, 447 aa, Artificial Sequence
  Synthetic (10_HeavyChain)
QVQLVQSGAEVKKPGSSVKVSCKASGGTFSSHYMHWVRQAPGQGLEWMGWISPYLGSTNYAQKFQGRVTITADESTSTAYMELSSLRSEDTAVYYCARDETGSTYGAFDYWGQGTLVTVSSASTKGPSVFPLAPCSRSTSESTAALGCLVKDYFPEPVTVSWNSGALTSGVHTFPAVLQSSGLYSLSSVVTVPSSSLGTKTYTCNVDHKPSNTKVDKRVESKYGPPCPPCPAPEAAGGPSVFLFPPKPKDTLMISRTPEVTCVVVDVSQEDPEVQFNWYVDGVEVHNAKTKPREEQFNSTYRVVSVLTVLHQDWLNGKEYKCKVSNKGLPSSIEKTISKAKGQPREPQVYTLPPSQEEMTKNQVSLTCLVKGFYPSDIAVEWESNGQPENNYKTTPPVLDSDGSFFLYSRLTVDKSRWQEGNVFSCSVMHEALHNHYTQKSLSLSLG

SEQ ID NO: 73 - protein, 11 aa, Artificial Sequence
  Synthetic (11_CDR-L1)
RASQSISNYLN

SEQ ID NO: 74 - protein, 7 aa, Artificial Sequence
  Synthetic (11_CDR-L2)
DASTLQS

SEQ ID NO: 75 - protein, 9 aa, Artificial Sequence
  Synthetic (11_CDR-L3)
QQSYSFPWT

SEQ ID NO: 76 - protein, 5 aa, Artificial Sequence
  Synthetic (11_CDR-H1)
SYYVH

SEQ ID NO: 77 - protein, 17 aa, Artificial Sequence
  Synthetic (11_CDR-H2)
WISPYSGGTNYAQKFQG

SEQ ID NO: 78 - protein, 12 aa, Artificial Sequence
  Synthetic (11_CDR-H3)
DYYVSAYGAFDY

SEQ ID NO: 79 - protein, 107 aa, Artificial Sequence
  Synthetic (11_LightChain_VariableRegion)
DIQMTQSPSSLSASVGDRVTITCRASQSISNYLNWYQQKPGKAPKLLIYDASTLQSGVPSRFSGSGSGTDFTLTISSLQPEDFATYYCQQSYSFPWTFGQGTKVEIK

SEQ ID NO: 80 - DNA, 321 bp, Artificial Sequence
  Synthetic (11_LightChain_VariableRegion_gene)
gacattcaaatgacgcagagtccctcctcactgagtgctagcgtgggcgatcgtgtgacaattacttgtcgcgctagccagtctatctctaattacctgaactggtatcagcagaaaccgggcaaggcgccaaaattgctgatttacgatgcatccactctgcagtctggtgtaccgtcccgtttctctggcagcggttctggtacggattttaccctgaccatctcaagcctccagcctgaagattttgccacctattattgtcagcaatcttactcttttccgtggacgttcgggcagggaactaaagtggaaattaaa

SEQ ID NO: 81 - protein, 121 aa, Artificial Sequence
  Synthetic (11_HeavyChain_VariableRegion)
QVQLVQSGAEVKKPGSSVKVSCKASGGTFSSYYVHWVRQAPGQGLEWMGWISPYSGGTNYAQKFQGRVTITADESTSTAYMELSSLRSEDTAVYYCARDYYVSAYGAFDYWGQGTLVTVSS

SEQ ID NO: 82 - DNA, 363 bp, Artificial Sequence
  Synthetic (11_HeavyChain_VariableRegion_gene)
caagttcagctggtccagagcggcgcagaggtgaagaagcccggcagttctgttaaggtttcctgcaaagcctcaggcgggacttttagttcttactacgttcattgggtgcggcaggcgcccggccagggtctcgaatggatggggtggatttctccatactctggtggtaccaactatgcacaaaaattccaaggccgcgtaactattaccgccgacgaatcaacctccaccgcctacatggaactcagctctctgaggtcagaagacacggccgtctattattgcgccagagattactacgtttctgcatacggtgcattcgattactggggtcagggtactctggttaccgtctcatcg

SEQ ID NO: 83 - protein, 214 aa, Artificial Sequence
  Synthetic (11_LightChain_Kappa)
DIQMTQSPSSLSASVGDRVTITCRASQSISNYLNWYQQKPGKAPKLLIYDASTLQSGVPSRFSGSGSGTDFTLTISSLQPEDFATYYCQQSYSFPWTFGQGTKVEIKRTVAAPSVFIFPPSDEQLKSGTASVVCLLNNFYPREAKVQWKVDNALQSGNSQESVTEQDSKDSTYSLSSTLTLSKADYEKHKVYACEVTHQGLSSPVTKSFNRGEC

SEQ ID NO: 84 - protein, 447 aa, Artificial Sequence
  Synthetic (11_HeavyChain)
QVQLVQSGAEVKKPGSSVKVSCKASGGTFSSYYVHWVRQAPGQGLEWMGWISPYSGGTNYAQKFQGRVTITADESTSTAYMELSSLRSEDTAVYYCARDYYVSAYGAFDYWGQGTLVTVSSASTKGPSVFPLAPCSRSTSESTAALGCLVKDYFPEPVTVSWNSGALTSGVHTFPAVLQSSGLYSLSSVVTVPSSSLGTKTYTCNVDHKPSNTKVDKRVESKYGPPCPPCPAPEAAGGPSVFLFPPKPKDTLMISRTPEVTCVVVDVSQEDPEVQFNWYVDGVEVHNAKTKPREEQFNSTYRVVSVLTVLHQDWLNGKEYKCKVSNKGLPSSIEKTISKAKGQPREPQVYTLPPSQEEMTKNQVSLTCLVKGFYPSDIAVEWESNGQPENNYKTTPPVLDSDGSFFLYSRLTVDKSRWQEGNVFSCSVMHEALHNHYTQKSLSLSLG

SEQ ID NO: 85 - protein, 11 aa, Artificial Sequence
  Synthetic (12_CDR-L1)
RASQDISNYLN

SEQ ID NO: 86 - protein, 7 aa, Artificial Sequence
  Synthetic (12_CDR-L2)
ATSSLQS

SEQ ID NO: 87 - protein, 9 aa, Artificial Sequence
  Synthetic (12_CDR-L3)
QQSYSFPWT

SEQ ID NO: 88 - protein, 5 aa, Artificial Sequence
  Synthetic (12_CDR-H1)
SYDIH

SEQ ID NO: 89 - protein, 17 aa, Artificial Sequence
  Synthetic (12_CDR-H2)
RIVPYLGVTNYAQKFQG

SEQ ID NO: 90 - protein, 12 aa, Artificial Sequence
  Synthetic (12_CDR-H3)
RQSQSSVYAFDI

SEQ ID NO: 91 - protein, 107 aa, Artificial Sequence
  Synthetic (12_LightChain_VariableRegion)
DIQMTQSPSSLSASVGDRVTITCRASQDISNYLNWYQQKPGKAPKLLIYATSSLQSGVPSRFSGSGSGTDFTLTISSLQPEDFATYYCQQSYSFPWTFGQGTKVEIK

SEQ ID NO: 92 - DNA, 321 bp, Artificial Sequence
  Synthetic (12_LightChain_VariableRegion_gene)
gacattcaaatgacgcagagtccctcctcactgagtgctagcgtgggcgatcgtgtgacaattacttgtcgcgctagccaggatatctctaattacctgaactggtatcagcagaaaccgggcaaggcgccaaaattgctgatttacgcaacttcctctctgcagtctggtgtaccgtcccgtttctctggcagcggttctggtacggattttaccctgaccatctcaagcctccagcctgaagattttgccacctattattgtcagcaatcttactcttttccgtggacgttcgggcagggaactaaagtggaaattaaa

SEQ ID NO: 93 - protein, 121 aa, Artificial Sequence
  Synthetic (12_HeavyChain_VariableRegion)
QVQLVQSGAEVKKPGSSVKVSCKASGGTFSSYDIHWVRQAPGQGLEWMGRIVPYLGVTNYAQKFQGRVTITADESTSTAYMELSSLRSEDTAVYYCARRQSQSSVYAFDIWGQGTLVTVSS

SEQ ID NO: 94 - DNA, 363 bp, Artificial Sequence
  Synthetic (12_HeavyChain_VariableRegion_gene)
caagttcagctggtccagagcggcgcagaggtgaagaagcccggcagttctgttaaggtttcctgcaaagcctcaggcgggacttttagttcttacgatatccattgggtgcggcaggcgcccggccagggtctcgaatggatggggcgtattgttccatacctgggtgttaccaactatgcacaaaaattccaaggccgcgtaactattaccgccgacgaatcaacctccaccgcctacatggaactcagctctctgaggtcagaagacacggccgtctattattgcgccagacgtcagtctcagtcttctgtttacgcattcgatatctggggtcagggcactttagtgaccgtctcatcg

SEQ ID NO: 95 - protein, 214 aa, Artificial Sequence
  Synthetic (12_LightChain_Kappa)
DIQMTQSPSSLSASVGDRVTITCRASQDISNYLNWYQQKPGKAPKLLIYATSSLQSGVPSRFSGSGSGTDFTLTISSLQPEDFATYYCQQSYSFPWTFGQGTKVEIKRTVAAPSVFIFPPSDEQLKSGTASVVCLLNNFYPREAKVQWKVDNALQSGNSQESVTEQDSKDSTYSLSSTLTLSKADYEKHKVYACEVTHQGLSSPVTKSFNRGEC

SEQ ID NO: 96 - protein, 447 aa, Artificial Sequence
  Synthetic (12_HeavyChain)
QVQLVQSGAEVKKPGSSVKVSCKASGGTFSSYDIHWVRQAPGQGLEWMGRIVPYLGVTNYAQKFQGRVTITADESTSTAYMELSSLRSEDTAVYYCARRQSQSSVYAFDIWGQGTLVTVSSASTKGPSVFPLAPCSRSTSESTAALGCLVKDYFPEPVTVSWNSGALTSGVHTFPAVLQSSGLYSLSSVVTVPSSSLGTKTYTCNVDHKPSNTKVDKRVESKYGPPCPPCPAPEAAGGPSVFLFPPKPKDTLMISRTPEVTCVVVDVSQEDPEVQFNWYVDGVEVHNAKTKPREEQFNSTYRVVSVLTVLHQDWLNGKEYKCKVSNKGLPSSIEKTISKAKGQPREPQVYTLPPSQEEMTKNQVSLTCLVKGFYPSDIAVEWESNGQPENNYKTTPPVLDSDGSFFLYSRLTVDKSRWQEGNVFSCSVMHEALHNHYTQKSLSLSLG

SEQ ID NO: 97 - protein, 11 aa, Artificial Sequence
  Synthetic (13_CDR-L1)
RASQSISNYLN

SEQ ID NO: 98 - protein, 7 aa, Artificial Sequence
  Synthetic (13_CDR-L2)
AASRLQS

SEQ ID NO: 99 - protein, 9 aa, Artificial Sequence
  Synthetic (13_CDR-L3)
QQSYSFPFT

SEQ ID NO: 100 - protein, 5 aa, Artificial Sequence
  Synthetic (13_CDR-H1)
GYYIH

SEQ ID NO: 101 - protein, 17 aa, Artificial Sequence
  Synthetic (13_CDR-H2)
WISPSSGGTIYAQKFQG

SEQ ID NO: 102 - protein, 12 aa, Artificial Sequence
  Synthetic (13_CDR-H3)
DISVRVVQAFDY

SEQ ID NO: 103 - protein, 107 aa, Artificial Sequence
  Synthetic (13_LightChain_VariableRegion)
DIQMTQSPSSLSASVGDRVTITCRASQSISNYLNWYQQKPGKAPKLLIYAASRLQSGVPSRFSGSGSGTDFTLTISSLQPEDFATYYCQQSYSFPFTFGQGTKVEIK

SEQ ID NO: 104 - DNA, 321 bp, Artificial Sequence
  Synthetic (13_LightChain_VariableRegion_gene)
gacattcaaatgacgcagagtccctcctcactgagtgctagcgtgggcgatcgtgtgacaattacttgtcgcgctagccagtctatctctaattacctgaactggtatcagcagaaaccgggcaaggcgccaaaattgctgatttacgcagcatcccgtctgcagtctggtgtaccgtcccgtttctctggcagcggttctggtacggattttaccctgaccatctcaagcctccagcctgaagattttgccacctattattgtcagcaatcttactcttttccgtttacgttcgggcagggaactaaagtggaaattaaa

SEQ ID NO: 105 - protein, 121 aa, Artificial Sequence
  Synthetic (13_HeavyChain_VariableRegion)
QVQLVQSGAEVKKPGSSVKVSCKASGGTFSGYYIHWVRQAPGQGLEWMGWISPSSGGTIYAQKFQGRVTITADESTSTAYMELSSLRSEDTAVYYCARDISVRVVQAFDYWGQGTLVTVSS

SEQ ID NO: 106 - DNA, 363 bp, Artificial Sequence
  Synthetic (13_HeavyChain_VariableRegion_gene)
caagttcagctggtccagagcggcgcagaggtgaagaagcccggcagttctgttaaggtttcctgcaaagcctcaggcgggacttttagtggttactacatccattgggtgcggcaggcgcccggccagggtctcgaatggatggggtggatttctccatcttctggtggtaccatctatgcacaaaaattccaaggccgcgtaactattaccgccgacgaatcaacctccaccgcctacatggaactcagctctctgaggtcagaagacacggccgtctattattgcgccagagatatctctgttcgtgttgttcaggcattcgattactggggtcagggtactctggttaccgtctcatcg

SEQ ID NO: 107 - protein, 214 aa, Artificial Sequence
  Synthetic (13_LightChain_Kappa)
DIQMTQSPSSLSASVGDRVTITCRASQSISNYLNWYQQKPGKAPKLLIYAASRLQSGVPSRFSGSGSGTDFTLTISSLQPEDFATYYCQQSYSFPFTFGQGTKVEIKRTVAAPSVFIFPPSDEQLKSGTASVVCLLNNFYPREAKVQWKVDNALQSGNSQESVTEQDSKDSTYSLSSTLTLSKADYEKHKVYACEVTHQGLSSPVTKSFNRGEC

SEQ ID NO: 108 - protein, 447 aa, Artificial Sequence
  Synthetic (13_HeavyChain)
QVQLVQSGAEVKKPGSSVKVSCKASGGTFSGYYIHWVRQAPGQGLEWMGWISPSSGGTIYAQKFQGRVTITADESTSTAYMELSSLRSEDTAVYYCARDISVRVVQAFDYWGQGTLVTVSSASTKGPSVFPLAPCSRSTSESTAALGCLVKDYFPEPVTVSWNSGALTSGVHTFPAVLQSSGLYSLSSVVTVPSSSLGTKTYTCNVDHKPSNTKVDKRVESKYGPPCPPCPAPEAAGGPSVFLFPPKPKDTLMISRTPEVTCVVVDVSQEDPEVQFNWYVDGVEVHNAKTKPREEQFNSTYRVVSVLTVLHQDWLNGKEYKCKVSNKGLPSSIEKTISKAKGQPREPQVYTLPPSQEEMTKNQVSLTCLVKGFYPSDIAVEWESNGQPENNYKTTPPVLDSDGSFFLYSRLTVDKSRWQEGNVFSCSVMHEALHNHYTQKSLSLSLG

SEQ ID NO: 109 - protein, 11 aa, Artificial Sequence
  Synthetic (14_CDR-L1)
RASQSISNYLN

SEQ ID NO: 110 - protein, 7 aa, Artificial Sequence
  Synthetic (14_CDR-L2)
ATSNLQS

SEQ ID NO: 111 - protein, 9 aa, Artificial Sequence
  Synthetic (14_CDR-L3)
QQSYSFPWT

SEQ ID NO: 112 - protein, 5 aa, Artificial Sequence
  Synthetic (14_CDR-H1)
SYYMH

SEQ ID NO: 113 - protein, 17 aa, Artificial Sequence
  Synthetic (14_CDR-H2)
WISPYLGITNYAQKFQG

SEQ ID NO: 114 - protein, 12 aa, Artificial Sequence
  Synthetic (14_CDR-H3)
AGYQQAQYWFDY

SEQ ID NO: 115 - protein, 107 aa, Artificial Sequence
  Synthetic (14_LightChain_VariableRegion)
DIQMTQSPSSLSASVGDRVTITCRASQSISNYLNWYQQKPGKAPKLLIYATSNLQSGVPSRFSGSGSGTDFTLTISSLQPEDFATYYCQQSYSFPWTFGQGTKVEIK

SEQ ID NO: 116 - DNA, 321 bp, Artificial Sequence
  Synthetic (14_LightChain_VariableRegion_gene)
gacattcaaatgacgcagagtccctcctcactgagtgctagcgtgggcgatcgtgtgacaattacttgtcgcgctagccagtctatctctaattacctgaactggtatcagcagaaaccgggcaaggcgccaaaattgctgatttacgcaacttccaatctgcagtctggtgtaccgtcccgtttctctggcagcggttctggtacggattttaccctgaccatctcaagcctccagcctgaagattttgccacctattattgtcagcaatcttactcttttccgtggacgttcgggcagggaactaaagtggaaattaaa

SEQ ID NO: 117 - protein, 121 aa, Artificial Sequence
  Synthetic (14_HeavyChain_VariableRegion)
QVQLVQSGAEVKKPGSSVKVSCKASGGTFSSYYMHWVRQAPGQGLEWMGWISPYLGITNYAQKFQGRVTITADESTSTAYMELSSLRSEDTAVYYCARAGYQQAQYWFDYWGQGTLVTVSS

SEQ ID NO: 118 - DNA, 363 bp, Artificial Sequence
  Synthetic (14_HeavyChain_VariableRegion_gene)
caagttcagctggtccagagcggcgcagaggtgaagaagcccggcagttctgttaaggtttcctgcaaagcctcaggcgggacttttagttcttactacatgcattgggtgcggcaggcgcccggccagggtctcgaatggatggggtggatttctccatacctgggtatcaccaactatgcacaaaaattccaaggccgcgtaactattaccgccgacgaatcaacctccaccgcctacatggaactcagctctctgaggtcagaagacacggccgtctattattgcgccagagcaggttaccagcaggcacagtactggttcgattactggggtcagggcactttagtgaccgtctcatcg

SEQ ID NO: 119 - protein, 214 aa, Artificial Sequence
  Synthetic (14_LightChain_Kappa)
DIQMTQSPSSLSASVGDRVTITCRASQSISNYLNWYQQKPGKAPKLLIYATSNLQSGVPSRFSGSGSGTDFTLTISSLQPEDFATYYCQQSYSFPWTFGQGTKVEIKRTVAAPSVFIFPPSDEQLKSGTASVVCLLNNFYPREAKVQWKVDNALQSGNSQESVTEQDSKDSTYSLSSTLTLSKADYEKHKVYACEVTHQGLSSPVTKSFNRGEC

SEQ ID NO: 120 - protein, 447 aa, Artificial Sequence
  Synthetic (14_HeavyChain)
QVQLVQSGAEVKKPGSSVKVSCKASGGTFSSYYMHWVRQAPGQGLEWMGWISPYLGITNYAQKFQGRVTITADESTSTAYMELSSLRSEDTAVYYCARAGYQQAQYWFDYWGQGTLVTVSSASTKGPSVFPLAPCSRSTSESTAALGCLVKDYFPEPVTVSWNSGALTSGVHTFPAVLQSSGLYSLSSVVTVPSSSLGTKTYTCNVDHKPSNTKVDKRVESKYGPPCPPCPAPEAAGGPSVFLFPPKPKDTLMISRTPEVTCVVVDVSQEDPEVQFNWYVDGVEVHNAKTKPREEQFNSTYRVVSVLTVLHQDWLNGKEYKCKVSNKGLPSSIEKTISKAKGQPREPQVYTLPPSQEEMTKNQVSLTCLVKGFYPSDIAVEWESNGQPENNYKTTPPVLDSDGSFFLYSRLTVDKSRWQEGNVFSCSVMHEALHNHYTQKSLSLSLG

SEQ ID NO: 121 - protein, 11 aa, Artificial Sequence
  Synthetic (15_CDR-L1)
RASQSISNYLN

SEQ ID NO: 122 - protein, 7 aa, Artificial Sequence
  Synthetic (15_CDR-L2)
ATSSLQS

SEQ ID NO: 123 - protein, 9 aa, Artificial Sequence
  Synthetic (15_CDR-L3)
QQSYSFPYT

SEQ ID NO: 124 - protein, 5 aa, Artificial Sequence
  Synthetic (15_CDR-H1)
SYAMS

SEQ ID NO: 125 - protein, 17 aa, Artificial Sequence
  Synthetic (15_CDR-H2)
WIIPISGTTNYAQKFQG

SEQ ID NO: 126 - protein, 10 aa, Artificial Sequence
  Synthetic (15_CDR-H3)
QHSVGSVFDY

SEQ ID NO: 127 - protein, 107 aa, Artificial Sequence
  Synthetic (15_LightChain_VariableRegion)
DIQMTQSPSSLSASVGDRVTITCRASQSISNYLNWYQQKPGKAPKLLIYATSSLQSGVPSRFSGSGSGTDFTLTISSLQPEDFATYYCQQSYSFPYTFGQGTKVEIK

SEQ ID NO: 128 - DNA, 321 bp, Artificial Sequence
  Synthetic (15_LightChain_VariableRegion_gene)
gacattcaaatgacgcagagtccctcctcactgagtgctagcgtgggcgatcgtgtgacaattacttgtcgcgctagccagtctatctctaattacctgaactggtatcagcagaaaccgggcaaggcgccaaaattgctgatttacgcaacttcctctctgcagtctggtgtaccgtcccgtttctctggcagcggttctggtacggattttaccctgaccatctcaagcctccagcctgaagattttgccacctattattgtcagcaatcttactcttttccgtacacgttcgggcagggaactaaagtggaaattaaa

SEQ ID NO: 129 - protein, 119 aa, Artificial Sequence
  Synthetic (15_HeavyChain_VariableRegion)
QVQLVQSGAEVKKPGSSVKVSCKASGGTFSSYAMSWVRQAPGQGLEWMGWIIPISGTTNYAQKFQGRVTITADESTSTAYMELSSLRSEDTAVYYCARQHSVGSVFDYWGQGTLVTVSS

SEQ ID NO: 130 - DNA, 357 bp, Artificial Sequence
  Synthetic (15_HeavyChain_VariableRegion_gene)
caagttcagctggtccagagcggcgcagaggtgaagaagcccggcagttctgttaaggtttcctgcaaagcctcaggcgggacttttagttcttacgcaatgtcttgggtgcggcaggcgcccggccagggtctcgaatggatggggtggattatcccaatctctggtaccaccaactatgcacaaaaattccaaggccgcgtaactattaccgccgacgaatcaacctccaccgcctacatggaactcagctctctgaggtcagaagacacggccgtctattattgcgccagacagcattctgttggttctgttttcgattactggggtcagggtactctggttaccgtctcatcg

SEQ ID NO: 131 - protein, 214 aa, Artificial Sequence
  Synthetic (15_LightChain_Kappa)
DIQMTQSPSSLSASVGDRVTITCRASQSISNYLNWYQQKPGKAPKLLIYATSSLQSGVPSRFSGSGSGTDFTLTISSLQPEDFATYYCQQSYSFPYTFGQGTKVEIKRTVAAPSVFIFPPSDEQLKSGTASVVCLLNNFYPREAKVQWKVDNALQSGNSQESVTEQDSKDSTYSLSSTLTLSKADYEKHKVYACEVTHQGLSSPVTKSFNRGEC

SEQ ID NO: 132 - protein, 445 aa, Artificial Sequence
  Synthetic (15_HeavyChain)
QVQLVQSGAEVKKPGSSVKVSCKASGGTFSSYAMSWVRQAPGQGLEWMGWIIPISGTTNYAQKFQGRVTITADESTSTAYMELSSLRSEDTAVYYCARQHSVGSVFDYWGQGTLVTVSSASTKGPSVFPLAPCSRSTSESTAALGCLVKDYFPEPVTVSWNSGALTSGVHTFPAVLQSSGLYSLSSVVTVPSSSLGTKTYTCNVDHKPSNTKVDKRVESKYGPPCPPCPAPEAAGGPSVFLFPPKPKDTLMISRTPEVTCVVVDVSQEDPEVQFNWYVDGVEVHNAKTKPREEQFNSTYRVVSVLTVLHQDWLNGKEYKCKVSNKGLPSSIEKTISKAKGQPREPQVYTLPPSQEEMTKNQVSLTCLVKGFYPSDIAVEWESNGQPENNYKTTPPVLDSDGSFFLYSRLTVDKSRWQEGNVFSCSVMHEALHNHYTQKSLSLSLG

SEQ ID NO: 133 - protein, 11 aa, Artificial Sequence
  Synthetic (16_CDR-L1)
RASQDISSWLN

SEQ ID NO: 134 - protein, 7 aa, Artificial Sequence
  Synthetic (16_CDR-L2)
AASSLQS

SEQ ID NO: 135 - protein, 9 aa, Artificial Sequence
  Synthetic (16_CDR-L3)
QQSYSFPWT

SEQ ID NO: 136 - protein, 5 aa, Artificial Sequence
  Synthetic (16_CDR-H1)
SYYMT

SEQ ID NO: 137 - protein, 17 aa, Artificial Sequence
  Synthetic (16_CDR-H2)
GISPILGVTNYAQKFQG

SEQ ID NO: 138 - protein, 12 aa, Artificial Sequence
  Synthetic (16_CDR-H3)
LLVGVSETYFDY

SEQ ID NO: 139 - protein, 107 aa, Artificial Sequence
  Synthetic (16_LightChain_VariableRegion)
DIQMTQSPSSLSASVGDRVTITCRASQDISSWLNWYQQKPGKAPKLLIYAASSLQSGVPSRFSGSGSGTDFTLTISSLQPEDFATYYCQQSYSFPWTFGQGTKVEIK

SEQ ID NO: 140 - DNA, 321 bp, Artificial Sequence
  Synthetic (16_LightChain_VariableRegion_gene)
gacattcaaatgacgcagagtccctcctcactgagtgctagcgtgggcgatcgtgtgacaattacttgtcgcgctagccaggatatctcttcttggctgaactggtatcagcagaaaccgggcaaggcgccaaaattgctgatttacgcagcatcctctctgcagtctggtgtaccgtcccgtttctctggcagcggttctggtacggattttaccctgaccatctcaagcctccagcctgaagattttgccacctattattgtcagcaatcttactcttttccgtggacgttcgggcagggaactaaagtggaaattaaa

SEQ ID NO: 141 - protein, 121 aa, Artificial Sequence
  Synthetic (16_HeavyChain_VariableRegion)
QVQLVQSGAEVKKPGSSVKVSCKASGGTFSSYYMTWVRQAPGQGLEWMGGISPILGVTNYAQKFQGRVTITADESTSTAYMELSSLRSEDTAVYYCARLLVGVSETYFDYWGQGTLVTVSS

SEQ ID NO: 142 - DNA, 363 bp, Artificial Sequence
  Synthetic (16_HeavyChain_VariableRegion_gene)
caagttcagctggtccagagcggcgcagaggtgaagaagcccggcagttctgttaaggtttcctgcaaagcctcaggcgggacttttagttcttactacatgacctgggtgcggcaggcgcccggccagggtctcgaatggatggggggtatttctccaatcctgggtgttaccaactatgcacaaaaattccaaggccgcgtaactattaccgccgacgaatcaacctccaccgcctacatggaactcagctctctgaggtcagaagacacggccgtctattattgcgccagactgctggttggtgtttctgaaacttacttcgattactggggtcagggtactctggttaccgtctcatcg

SEQ ID NO: 143 - protein, 214 aa, Artificial Sequence
  Synthetic (16_LightChain_Kappa)
DIQMTQSPSSLSASVGDRVTITCRASQDISSWLNWYQQKPGKAPKLLIYAASSLQSGVPSRFSGSGSGTDFTLTISSLQPEDFATYYCQQSYSFPWTFGQGTKVEIKRTVAAPSVFIFPPSDEQLKSGTASVVCLLNNFYPREAKVQWKVDNALQSGNSQESVTEQDSKDSTYSLSSTLTLSKADYEKHKVYACEVTHQGLSSPVTKSFNRGEC

SEQ ID NO: 144 - protein, 447 aa, Artificial Sequence
  Synthetic (16_HeavyChain)
QVQLVQSGAEVKKPGSSVKVSCKASGGTFSSYYMTWVRQAPGQGLEWMGGISPILGVTNYAQKFQGRVTITADESTSTAYMELSSLRSEDTAVYYCARLLVGVSETYFDYWGQGTLVTVSSASTKGPSVFPLAPCSRSTSESTAALGCLVKDYFPEPVTVSWNSGALTSGVHTFPAVLQSSGLYSLSSVVTVPSSSLGTKTYTCNVDHKPSNTKVDKRVESKYGPPCPPCPAPEAAGGPSVFLFPPKPKDTLMISRTPEVTCVVVDVSQEDPEVQFNWYVDGVEVHNAKTKPREEQFNSTYRVVSVLTVLHQDWLNGKEYKCKVSNKGLPSSIEKTISKAKGQPREPQVYTLPPSQEEMTKNQVSLTCLVKGFYPSDIAVEWESNGQPENNYKTTPPVLDSDGSFFLYSRLTVDKSRWQEGNVFSCSVMHEALHNHYTQKSLSLSLG

SEQ ID NO: 145 - protein, 11 aa, Artificial Sequence
  Synthetic (17_CDR-L1)
RASQSISNYLN

SEQ ID NO: 146 - protein, 7 aa, Artificial Sequence
  Synthetic (17_CDR-L2)
AASNMHS

SEQ ID NO: 147 - protein, 9 aa, Artificial Sequence
  Synthetic (17_CDR-L3)
QQSHSFPWT

SEQ ID NO: 148 - protein, 5 aa, Artificial Sequence
  Synthetic (17_CDR-H1)
TYAMS

SEQ ID NO: 149 - protein, 17 aa, Artificial Sequence
  Synthetic (17_CDR-H2)
GISPTLGIANYAQKFQG

SEQ ID NO: 150 - protein, 12 aa, Artificial Sequence
  Synthetic (17_CDR-H3)
VRYAGWTGYFDL

SEQ ID NO: 151 - protein, 107 aa, Artificial Sequence
  Synthetic (17_LightChain_VariableRegion)
DIQMTQSPSSLSASVGDRVTITCRASQSISNYLNWYQQKPGKAPKLLIYAASNMHSGVPSRFSGSGSGTDFTLTISSLQPEDFATYYCQQSHSFPWTFGQGTKVEIK

SEQ ID NO: 152 - DNA, 321 bp, Artificial Sequence
  Synthetic (17_LightChain_VariableRegion_gene)
gacattcaaatgacgcagagtccctcctcactgagtgctagcgtgggcgatcgtgtgacaattacttgtcgcgctagccagtctatctctaattacctgaactggtatcagcagaaaccgggcaaggcgccaaaattgctgatttacgcagcatccaatatgcactctggtgtaccgtcccgtttctctggcagcggttctggtacggattttaccctgaccatctcaagcctccagcctgaagattttgccacctattattgtcagcaatctcactcttttccgtggacgttcgggcagggaactaaagtggaaattaaa

SEQ ID NO: 153 - protein, 121 aa, Artificial Sequence
  Synthetic (17_HeavyChain_VariableRegion)
QVQLVQSGAEVKKPGSSVKVSCKASGGTFSTYAMSWVRQAPGQGLEWMGGISPTLGIANYAQKFQGRVTITADESTSTAYMELSSLRSEDTAVYYCARVRYAGWTGYFDLWGQGTLVTVSS

SEQ ID NO: 154 - DNA, 363 bp, Artificial Sequence
  Synthetic (17_HeavyChain_VariableRegion_gene)
caagttcagctggtccagagcggcgcagaggtgaagaagcccggcagttctgttaaggtttcctgcaaagcctcaggcgggacttttagtacctacgcaatgtcttgggtgcggcaggcgcccggccagggtctcgaatggatggggggtatttctccaaccctgggtatcgcaaactatgcacaaaaattccaaggccgcgtaactattaccgccgacgaatcaacctccaccgcctacatggaactcagctctctgaggtcagaagacacggccgtctattattgcgccagagttcgttacgcaggttggactggttacttcgatctgtggggtcagggtactctggttaccgtctcatcg

SEQ ID NO: 155 - protein, 214 aa, Artificial Sequence
  Synthetic (17_LightChain_Kappa)
DIQMTQSPSSLSASVGDRVTITCRASQSISNYLNWYQQKPGKAPKLLIYAASNMHSGVPSRFSGSGSGTDFTLTISSLQPEDFATYYCQQSHSFPWTFGQGTKVEIKRTVAAPSVFIFPPSDEQLKSGTASVVCLLNNFYPREAKVQWKVDNALQSGNSQESVTEQDSKDSTYSLSSTLTLSKADYEKHKVYACEVTHQGLSSPVTKSFNRGEC

SEQ ID NO: 156 - protein, 447 aa, Artificial Sequence
  Synthetic (17_HeavyChain)
QVQLVQSGAEVKKPGSSVKVSCKASGGTFSTYAMSWVRQAPGQGLEWMGGISPTLGIANYAQKFQGRVTITADESTSTAYMELSSLRSEDTAVYYCARVRYAGWTGYFDLWGQGTLVTVSSASTKGPSVFPLAPCSRSTSESTAALGCLVKDYFPEPVTVSWNSGALTSGVHTFPAVLQSSGLYSLSSVVTVPSSSLGTKTYTCNVDHKPSNTKVDKRVESKYGPPCPPCPAPEAAGGPSVFLFPPKPKDTLMISRTPEVTCVVVDVSQEDPEVQFNWYVDGVEVHNAKTKPREEQFNSTYRVVSVLTVLHQDWLNGKEYKCKVSNKGLPSSIEKTISKAKGQPREPQVYTLPPSQEEMTKNQVSLTCLVKGFYPSDIAVEWESNGQPENNYKTTPPVLDSDGSFFLYSRLTVDKSRWQEGNVFSCSVMHEALHNHYTQKSLSLSLG

SEQ ID NO: 157 - protein, 11 aa, Artificial Sequence
  Synthetic (18_CDR-L1)
RASQSISRWLN

SEQ ID NO: 158 - protein, 7 aa, Artificial Sequence
  Synthetic (18_CDR-L2)
AASRLQS

SEQ ID NO: 159 - protein, 9 aa, Artificial Sequence
  Synthetic (18_CDR-L3)
QQSESFPWT

SEQ ID NO: 160 - protein, 5 aa, Artificial Sequence
  Synthetic (18_CDR-H1)
SYDIN

SEQ ID NO: 161 - protein, 17 aa, Artificial Sequence
  Synthetic (18_CDR-H2)
WIIPTSGSTNYAQKFQG

SEQ ID NO: 162 - protein, 12 aa, Artificial Sequence
  Synthetic (18_CDR-H3)
DSQSSYIGYFDV

SEQ ID NO: 163 - protein, 107 aa, Artificial Sequence
  Synthetic (18_LightChain_VariableRegion)
DIQMTQSPSSLSASVGDRVTITCRASQSISRWLNWYQQKPGKAPKLLIYAASRLQSGVPSRFSGSGSGTDFTLTISSLQPEDFATYYCQQSESFPWTFGQGTKVEIK

SEQ ID NO: 164 - DNA, 321 bp, Artificial Sequence
  Synthetic (18_LightChain_VariableRegion_gene)
gacattcaaatgacgcagagtccctcctcactgagtgctagcgtgggcgatcgtgtgacaattacttgtcgcgctagccagtctatctctcgttggctgaactggtatcagcagaaaccgggcaaggcgccaaaattgctgatttacgcagcatcccgtctgcagtctggtgtaccgtcccgtttctctggcagcggttctggtacggattttaccctgaccatctcaagcctccagcctgaagattttgccacctattattgtcagcaatctgaatcttttccgtggacgttcgggcagggaactaaagtggaaattaaa

SEQ ID NO: 165 - protein, 121 aa, Artificial Sequence
  Synthetic (18_HeavyChain_VariableRegion)
QVQLVQSGAEVKKPGSSVKVSCKASGGTFSSYDINWVRQAPGQGLEWMGWIIPTSGSTNYAQKFQGRVTITADESTSTAYMELSSLRSEDTAVYYCARDSQSSYIGYFDVWGQGTLVTVSS

SEQ ID NO: 166 - DNA, 363 bp, Artificial Sequence
  Synthetic (18_HeavyChain_VariableRegion_gene)
caagttcagctggtccagagcggcgcagaggtgaagaagcccggcagttctgttaaggtttcctgcaaagcctcaggcgggacttttagttcttacgatatcaactgggtgcggcaggcgcccggccagggtctcgaatggatggggtggattatcccaacctctggttctaccaactatgcacaaaaattccaaggccgcgtaactattaccgccgacgaatcaacctccaccgcctacatggaactcagctctctgaggtcagaagacacggccgtctattattgcgccagagattctcagtcttcttacatcggttacttcgatgtttggggtcagggtactctggttaccgtctcatcg

SEQ ID NO: 167 - protein, 214 aa, Artificial Sequence
  Synthetic (18_LightChain_Kappa)
DIQMTQSPSSLSASVGDRVTITCRASQSISRWLNWYQQKPGKAPKLLIYAASRLQSGVPSRFSGSGSGTDFTLTISSLQPEDFATYYCQQSESFPWTFGQGTKVEIKRTVAAPSVFIFPPSDEQLKSGTASVVCLLNNFYPREAKVQWKVDNALQSGNSQESVTEQDSKDSTYSLSSTLTLSKADYEKHKVYACEVTHQGLSSPVTKSFNRGEC

SEQ ID NO: 168 - protein, 447 aa, Artificial Sequence
  Synthetic (18_HeavyChain)
QVQLVQSGAEVKKPGSSVKVSCKASGGTFSSYDINWVRQAPGQGLEWMGWIIPTSGSTNYAQKFQGRVTITADESTSTAYMELSSLRSEDTAVYYCARDSQSSYIGYFDVWGQGTLVTVSSASTKGPSVFPLAPCSRSTSESTAALGCLVKDYFPEPVTVSWNSGALTSGVHTFPAVLQSSGLYSLSSVVTVPSSSLGTKTYTCNVDHKPSNTKVDKRVESKYGPPCPPCPAPEAAGGPSVFLFPPKPKDTLMISRTPEVTCVVVDVSQEDPEVQFNWYVDGVEVHNAKTKPREEQFNSTYRVVSVLTVLHQDWLNGKEYKCKVSNKGLPSSIEKTISKAKGQPREPQVYTLPPSQEEMTKNQVSLTCLVKGFYPSDIAVEWESNGQPENNYKTTPPVLDSDGSFFLYSRLTVDKSRWQEGNVFSCSVMHEALHNHYTQKSLSLSLG

SEQ ID NO: 169 - protein, 11 aa, Artificial Sequence
  Synthetic (19_CDR-L1)
RASQSISNYLN

SEQ ID NO: 170 - protein, 7 aa, Artificial Sequence
  Synthetic (19_CDR-L2)
DTSSLQS

SEQ ID NO: 171 - protein, 9 aa, Artificial Sequence
  Synthetic (19_CDR-L3)
QQSYSTPYT

SEQ ID NO: 172 - protein, 5 aa, Artificial Sequence
  Synthetic (19_CDR-H1)
AYGIS

SEQ ID NO: 173 - protein, 17 aa, Artificial Sequence
  Synthetic (19_CDR-H2)
RIIPYLGTANYAQKFQG

SEQ ID NO: 174 - protein, 12 aa, Artificial Sequence
  Synthetic (19_CDR-H3)
LSYGIGYESFDV

SEQ ID NO: 175 - protein, 107 aa, Artificial Sequence
  Synthetic (19_LightChain_VariableRegion)
DIQMTQSPSSLSASVGDRVTITCRASQSISNYLNWYQQKPGKAPKLLIYDTSSLQSGVPSRFSGSGSGTDFTLTISSLQPEDFATYYCQQSYSTPYTFGQGTKVEIK

SEQ ID NO: 176 - DNA, 321 bp, Artificial Sequence
  Synthetic (19_LightChain_VariableRegion_gene)
gacattcaaatgacgcagagtccctcctcactgagtgctagcgtgggcgatcgtgtgacaattacttgtcgcgctagccagtctatctctaattacctgaactggtatcagcagaaaccgggcaaggcgccaaaattgctgatttacgatacttcctctctgcagtctggtgtaccgtcccgtttctctggcagcggttctggtacggattttaccctgaccatctcaagcctccagcctgaagattttgccacctattattgtcagcaatcttactctactccgtacacgttcgggcagggaactaaagtggaaattaaa

SEQ ID NO: 177 - protein, 121 aa, Artificial Sequence
  Synthetic (19_HeavyChain_VariableRegion)
QVQLVQSGAEVKKPGSSVKVSCKASGGTFSAYGISWVRQAPGQGLEWMGRIIPYLGTANYAQKFQGRVTITADESTSTAYMELSSLRSEDTAVYYCARLSYGIGYESFDVWGQGTLVTVSS

SEQ ID NO: 178 - DNA, 363 bp, Artificial Sequence
  Synthetic (19_HeavyChain_VariableRegion_gene)
caagttcagctggtccagagcggcgcagaggtgaagaagcccggcagttctgttaaggtttcctgcaaagcctcaggcgggacttttagtgcatacggtatctcttgggtgcggcaggcgcccggccagggtctcgaatggatggggcgtattatcccatacctgggtaccgcaaactatgcacaaaaattccaaggccgcgtaactattaccgccgacgaatcaacctccaccgcctacatggaactcagctctctgaggtcagaagacacggccgtctattattgcgccagactgtcttacggtatcggttacgaatctttcgatgtttggggtcagggcactttagtgaccgtctcatcg

SEQ ID NO: 179 - protein, 214 aa, Artificial Sequence
  Synthetic (19_LightChain_Kappa)
DIQMTQSPSSLSASVGDRVTITCRASQSISNYLNWYQQKPGKAPKLLIYDTSSLQSGVPSRFSGSGSGTDFTLTISSLQPEDFATYYCQQSYSTPYTFGQGTKVEIKRTVAAPSVFIFPPSDEQLKSGTASVVCLLNNFYPREAKVQWKVDNALQSGNSQESVTEQDSKDSTYSLSSTLTLSKADYEKHKVYACEVTHQGLSSPVTKSFNRGEC

SEQ ID NO: 180 - protein, 447 aa, Artificial Sequence
  Synthetic (19_HeavyChain)
QVQLVQSGAEVKKPGSSVKVSCKASGGTFSAYGISWVRQAPGQGLEWMGRIIPYLGTANYAQKFQGRVTITADESTSTAYMELSSLRSEDTAVYYCARLSYGIGYESFDVWGQGTLVTVSSASTKGPSVFPLAPCSRSTSESTAALGCLVKDYFPEPVTVSWNSGALTSGVHTFPAVLQSSGLYSLSSVVTVPSSSLGTKTYTCNVDHKPSNTKVDKRVESKYGPPCPPCPAPEAAGGPSVFLFPPKPKDTLMISRTPEVTCVVVDVSQEDPEVQFNWYVDGVEVHNAKTKPREEQFNSTYRVVSVLTVLHQDWLNGKEYKCKVSNKGLPSSIEKTISKAKGQPREPQVYTLPPSQEEMTKNQVSLTCLVKGFYPSDIAVEWESNGQPENNYKTTPPVLDSDGSFFLYSRLTVDKSRWQEGNVFSCSVMHEALHNHYTQKSLSLSLG

SEQ ID NO: 181 - protein, 11 aa, Artificial Sequence
  Synthetic (20_CDR-L1)
RASQSISSYLN

SEQ ID NO: 182 - protein, 7 aa, Artificial Sequence
  Synthetic (20_CDR-L2)
DTSTLQS

SEQ ID NO: 183 - protein, 9 aa, Artificial Sequence
  Synthetic (20_CDR-L3)
QQSYSFPWT

SEQ ID NO: 184 - protein, 5 aa, Artificial Sequence
  Synthetic (20_CDR-H1)
SYAMS

SEQ ID NO: 185 - protein, 17 aa, Artificial Sequence
  Synthetic (20_CDR-H2)
SISSSGGSTYYADSVKG

SEQ ID NO: 186 - protein, 12 aa, Artificial Sequence
  Synthetic (20_CDR-H3)
ELGGYGFSYFDY

SEQ ID NO: 187 - protein, 107 aa, Artificial Sequence
  Synthetic (20_LightChain_VariableRegion)
DIQMTQSPSSLSASVGDRVTITCRASQSISSYLNWYQQKPGKAPKLLIYDTSTLQSGVPSRFSGSGSGTDFTLTISSLQPEDFATYYCQQSYSFPWTFGQGTKVEIK

SEQ ID NO: 188 - DNA, 321 bp, Artificial Sequence
  Synthetic (20_LightChain_VariableRegion_gene)
gacattcaaatgacgcagagtccctcctcactgagtgctagcgtgggcgatcgtgtgacaattacttgtcgcgctagccagtctatctcttcttacctgaactggtatcagcagaaaccgggcaaggcgccaaaattgctgatttacgatacttccactctgcagtctggtgtaccgtcccgtttctctggcagcggttctggtacggattttaccctgaccatctcaagcctccagcctgaagattttgccacctattattgtcagcaatcttactcttttccgtggacgttcgggcagggaactaaagtggaaattaaa

SEQ ID NO: 189 - protein, 121 aa, Artificial Sequence
  Synthetic (20_HeavyChain_VariableRegion)
QVQLVQSGAEVKKPGSSVKVSCKASGGTFSSYAMSWVRQAPGQGLEWMGSISSSGGSTYYADSVKGRVTITADESTSTAYMELSSLRSEDTAVYYCARELGGYGFSYFDYWGQGTLVTVSS

SEQ ID NO: 190 - DNA, 363 bp, Artificial Sequence
  Synthetic (20_HeavyChain_VariableRegion_gene)
caagttcagctggtccagagcggcgcagaggtgaagaagcccggcagttctgttaaggtttcctgcaaagcctcaggcgggacttttagttcttatgcaatgtcttgggtgcggcaggcgcccggccagggtctcgaatggatggggtctatctcttcttctggtggttctacttactatgccgattcagtgaagggtcgcgtaactattaccgccgacgaatcaacctccaccgcctacatggaactcagctctctgaggtcagaagacacggccgtctattattgcgccagagaactgggtggttacggtttctcttacttcgattactggggtcagggcactttagtgaccgtctcatcg

SEQ ID NO: 191 - protein, 214 aa, Artificial Sequence
  Synthetic (20_LightChain_Kappa)
DIQMTQSPSSLSASVGDRVTITCRASQSISSYLNWYQQKPGKAPKLLIYDTSTLQSGVPSRFSGSGSGTDFTLTISSLQPEDFATYYCQQSYSFPWTFGQGTKVEIKRTVAAPSVFIFPPSDEQLKSGTASVVCLLNNFYPREAKVQWKVDNALQSGNSQESVTEQDSKDSTYSLSSTLTLSKADYEKHKVYACEVTHQGLSSPVTKSFNRGEC

SEQ ID NO: 192 - protein, 447 aa, Artificial Sequence
  Synthetic (20_HeavyChain)
QVQLVQSGAEVKKPGSSVKVSCKASGGTFSSYAMSWVRQAPGQGLEWMGSISSSGGSTYYADSVKGRVTITADESTSTAYMELSSLRSEDTAVYYCARELGGYGFSYFDYWGQGTLVTVSSASTKGPSVFPLAPCSRSTSESTAALGCLVKDYFPEPVTVSWNSGALTSGVHTFPAVLQSSGLYSLSSVVTVPSSSLGTKTYTCNVDHKPSNTKVDKRVESKYGPPCPPCPAPEAAGGPSVFLFPPKPKDTLMISRTPEVTCVVVDVSQEDPEVQFNWYVDGVEVHNAKTKPREEQFNSTYRVVSVLTVLHQDWLNGKEYKCKVSNKGLPSSIEKTISKAKGQPREPQVYTLPPSQEEMTKNQVSLTCLVKGFYPSDIAVEWESNGQPENNYKTTPPVLDSDGSFFLYSRLTVDKSRWQEGNVFSCSVMHEALHNHYTQKSLSLSLG

SEQ ID NO: 193 - protein, 11 aa, Artificial Sequence
  Synthetic (21_CDR-L1)
RASQSIRNYLN

SEQ ID NO: 194 - protein, 7 aa, Artificial Sequence
  Synthetic (21_CDR-L2)
ATSSLQS

SEQ ID NO: 195 - protein, 9 aa, Artificial Sequence
  Synthetic (21_CDR-L3)
QQSYSFPWT

SEQ ID NO: 196 - protein, 5 aa, Artificial Sequence
  Synthetic (21_CDR-H1)
DYAMS

SEQ ID NO: 197 - protein, 15 aa, Artificial Sequence
  Synthetic (21_CDR-H2)
GISGSDIYYADSVKG

SEQ ID NO: 198 - protein, 11 aa, Artificial Sequence
  Synthetic (21_CDR-H3)
AVSYWSYTFDY

SEQ ID NO: 199 - protein, 107 aa, Artificial Sequence
  Synthetic (21_LightChain_VariableRegion)
DIQMTQSPSSLSASVGDRVTITCRASQSIRNYLNWYQQKPGKAPKLLIYATSSLQSGVPSRFSGSGSGTDFTLTISSLQPEDFATYYCQQSYSFPWTFGQGTKVEIK

SEQ ID NO: 200 - DNA, 321 bp, Artificial Sequence
  Synthetic (21_LightChain_VariableRegion_gene)
gacattcaaatgacgcagagtccctcctcactgagtgctagcgtgggcgatcgtgtgacaattacttgtcgcgctagccagtctatccgtaattacctgaactggtatcagcagaaaccgggcaaggcgccaaaattgctgatttacgcaacttcctctctgcagtctggtgtaccgtcccgtttctctggcagcggttctggtacggattttaccctgaccatctcaagcctccagcctgaagattttgccacctattattgtcagcaatcttactcttttccgtggacgttcgggcagggaactaaagtggaaattaaa

SEQ ID NO: 201 - protein, 118 aa, Artificial Sequence
  Synthetic (21_HeavyChain_VariableRegion)
QVQLVQSGAEVKKPGSSVKVSCKASGGTFSDYAMSWVRQAPGQGLEWMGGISGSDIYYADSVKGRVTITADESTSTAYMELSSLRSEDTAVYYCARAVSYWSYTFDYWGQGTLVTVSS

SEQ ID NO: 202 - DNA, 354 bp, Artificial Sequence
  Synthetic (21_HeavyChain_VariableRegion_gene)
caagttcagctggtccagagcggcgcagaggtgaagaagcccggcagttctgttaaggtttcctgcaaagcctcaggcgggacttttagtgattatgcaatgtcttgggtgcggcaggcgcccggccagggtctcgaatggatggggggtatctctggttctgatatctactatgccgattcagtgaagggtcgcgtaactattaccgccgacgaatcaacctccaccgcctacatggaactcagctctctgaggtcagaagacacggccgtctattattgcgccagagcagtttcttactggtcttacacttttgattactggggtcagggcactttagtgaccgtctcatcg

SEQ ID NO: 203 - protein, 214 aa, Artificial Sequence
  Synthetic (21_LightChain_Kappa)
DIQMTQSPSSLSASVGDRVTITCRASQSIRNYLNWYQQKPGKAPKLLIYATSSLQSGVPSRFSGSGSGTDFTLTISSLQPEDFATYYCQQSYSFPWTFGQGTKVEIKRTVAAPSVFIFPPSDEQLKSGTASVVCLLNNFYPREAKVQWKVDNALQSGNSQESVTEQDSKDSTYSLSSTLTLSKADYEKHKVYACEVTHQGLSSPVTKSFNRGEC

SEQ ID NO: 204 - protein, 444 aa, Artificial Sequence
  Synthetic (21_HeavyChain)
QVQLVQSGAEVKKPGSSVKVSCKASGGTFSDYAMSWVRQAPGQGLEWMGGISGSDIYYADSVKGRVTITADESTSTAYMELSSLRSEDTAVYYCARAVSYWSYTFDYWGQGTLVTVSSASTKGPSVFPLAPCSRSTSESTAALGCLVKDYFPEPVTVSWNSGALTSGVHTFPAVLQSSGLYSLSSVVTVPSSSLGTKTYTCNVDHKPSNTKVDKRVESKYGPPCPPCPAPEAAGGPSVFLFPPKPKDTLMISRTPEVTCVVVDVSQEDPEVQFNWYVDGVEVHNAKTKPREEQFNSTYRVVSVLTVLHQDWLNGKEYKCKVSNKGLPSSIEKTISKAKGQPREPQVYTLPPSQEEMTKNQVSLTCLVKGFYPSDIAVEWESNGQPENNYKTTPPVLDSDGSFFLYSRLTVDKSRWQEGNVFSCSVMHEALHNHYTQKSLSLSLG

SEQ ID NO: 205 - protein, 11 aa, Artificial Sequence
  Synthetic (22_CDR-L1)
RASQSIGSYLN

SEQ ID NO: 206 - protein, 7 aa, Artificial Sequence
  Synthetic (22_CDR-L2)
DASTLQS

SEQ ID NO: 207 - protein, 9 aa, Artificial Sequence
  Synthetic (22_CDR-L3)
QQSYSFPWT

SEQ ID NO: 208 - protein, 5 aa, Artificial Sequence
  Synthetic (22_CDR-H1)
SYAMH

SEQ ID NO: 209 - protein, 17 aa, Artificial Sequence
  Synthetic (22_CDR-H2)
GISSSGGTTYYADSVKG

SEQ ID NO: 210 - protein, 12 aa, Artificial Sequence
  Synthetic (22_CDR-H3)
ALGVVGGTWFDY

SEQ ID NO: 211 - protein, 107 aa, Artificial Sequence
  Synthetic (22_LightChain_VariableRegion)
DIQMTQSPSSLSASVGDRVTITCRASQSIGSYLNWYQQKPGKAPKLLIYDASTLQSGVPSRFSGSGSGTDFTLTISSLQPEDFATYYCQQSYSFPWTFGQGTKVEIK

SEQ ID NO: 212 - DNA, 321 bp, Artificial Sequence
  Synthetic (22_LightChain_VariableRegion_gene)
gacattcaaatgacgcagagtccctcctcactgagtgctagcgtgggcgatcgtgtgacaattacttgtcgcgctagccagtctatcggttcttacctgaactggtatcagcagaaaccgggcaaggcgccaaaattgctgatttacgatgcatccactctgcagtctggtgtaccgtcccgtttctctggcagcggttctggtacggattttaccctgaccatctcaagcctccagcctgaagattttgccacctattattgtcagcaatcttactcttttccgtggacgttcgggcagggaactaaagtggaaattaaa

SEQ ID NO: 213 - protein, 121 aa, Artificial Sequence
  Synthetic (22_HeavyChain_VariableRegion)
QVQLVQSGAEVKKPGSSVKVSCKASGGTFSSYAMHWVRQAPGQGLEWMGGISSSGGTTYYADSVKGRVTITADESTSTAYMELSSLRSEDTAVYYCARALGVVGGTWFDYWGQGTLVTVSS

SEQ ID NO: 214 - DNA, 363 bp, Artificial Sequence
  Synthetic (22_HeavyChain_VariableRegion_gene)
caagttcagctggtccagagcggcgcagaggtgaagaagcccggcagttctgttaaggtttcctgcaaagcctcaggcgggacttttagttcttatgcaatgcactgggtgcggcaggcgcccggccagggtctcgaatggatggggggtatctcttcttctggtggtactacttactatgccgattcagtgaagggtcgcgtaactattaccgccgacgaatcaacctccaccgcctacatggaactcagctctctgaggtcagaagacacggccgtctattattgcgccagagcactgggtgttgttggtggtacttggttcgattactggggtcagggcactttagtgaccgtctcatcg

SEQ ID NO: 215 - protein, 214 aa, Artificial Sequence
  Synthetic (22_LightChain_Kappa)
DIQMTQSPSSLSASVGDRVTITCRASQSIGSYLNWYQQKPGKAPKLLIYDASTLQSGVPSRFSGSGSGTDFTLTISSLQPEDFATYYCQQSYSFPWTFGQGTKVEIKRTVAAPSVFIFPPSDEQLKSGTASVVCLLNNFYPREAKVQWKVDNALQSGNSQESVTEQDSKDSTYSLSSTLTLSKADYEKHKVYACEVTHQGLSSPVTKSFNRGEC

SEQ ID NO: 216 - protein, 447 aa, Artificial Sequence
  Synthetic (22_HeavyChain)
QVQLVQSGAEVKKPGSSVKVSCKASGGTFSSYAMHWVRQAPGQGLEWMGGISSSGGTTYYADSVKGRVTITADESTSTAYMELSSLRSEDTAVYYCARALGVVGGTWFDYWGQGTLVTVSSASTKGPSVFPLAPCSRSTSESTAALGCLVKDYFPEPVTVSWNSGALTSGVHTFPAVLQSSGLYSLSSVVTVPSSSLGTKTYTCNVDHKPSNTKVDKRVESKYGPPCPPCPAPEAAGGPSVFLFPPKPKDTLMISRTPEVTCVVVDVSQEDPEVQFNWYVDGVEVHNAKTKPREEQFNSTYRVVSVLTVLHQDWLNGKEYKCKVSNKGLPSSIEKTISKAKGQPREPQVYTLPPSQEEMTKNQVSLTCLVKGFYPSDIAVEWESNGQPENNYKTTPPVLDSDGSFFLYSRLTVDKSRWQEGNVFSCSVMHEALHNHYTQKSLSLSLG

SEQ ID NO: 217 - protein, 11 aa, Artificial Sequence
  Synthetic (23_CDR-L1)
RASQSISNYLN

SEQ ID NO: 218 - protein, 7 aa, Artificial Sequence
  Synthetic (23_CDR-L2)
DTSTLQS

SEQ ID NO: 219 - protein, 9 aa, Artificial Sequence
  Synthetic (23_CDR-L3)
QQSYSFPWT

SEQ ID NO: 220 - protein, 5 aa, Artificial Sequence
  Synthetic (23_CDR-H1)
DYAMH

SEQ ID NO: 221 - protein, 17 aa, Artificial Sequence
  Synthetic (23_CDR-H2)
AISGSGGYTHYADSVKG

SEQ ID NO: 222 - protein, 12 aa, Artificial Sequence
  Synthetic (23_CDR-H3)
SATFGVWETFDV

SEQ ID NO: 223 - protein, 107 aa, Artificial Sequence
  Synthetic (23_LightChain_VariableRegion)
DIQMTQSPSSLSASVGDRVTITCRASQSISNYLNWYQQKPGKAPKLLIYDTSTLQSGVPSRFSGSGSGTDFTLTISSLQPEDFATYYCQQSYSFPWTFGQGTKVEIK

SEQ ID NO: 224 - DNA, 321 bp, Artificial Sequence
  Synthetic (23_LightChain_VariableRegion_gene)
gacattcaaatgacgcagagtccctcctcactgagtgctagcgtgggcgatcgtgtgacaattacttgtcgcgctagccagtctatctctaattacctgaactggtatcagcagaaaccgggcaaggcgccaaaattgctgatttacgatacttccactctgcagtctggtgtaccgtcccgtttctctggcagcggttctggtacggattttaccctgaccatctcaagcctccagcctgaagattttgccacctattattgtcagcaatcttactcttttccgtggacgttcgggcagggaactaaagtggaaattaaa

SEQ ID NO: 225 - protein, 121 aa, Artificial Sequence
  Synthetic (23_HeavyChain_VariableRegion)
QVQLVQSGAEVKKPGSSVKVSCKASGGTFSDYAMHWVRQAPGQGLEWMGAISGSGGYTHYADSVKGRVTITADESTSTAYMELSSLRSEDTAVYYCARSATFGVWETFDVWGQGTLVTVSS

SEQ ID NO: 226 - DNA, 363 bp, Artificial Sequence
  Synthetic (23_HeavyChain_VariableRegion_gene)
caagttcagctggtccagagcggcgcagaggtgaagaagcccggcagttctgttaaggtttcctgcaaagcctcaggcgggacttttagtgattatgcaatgcactgggtgcggcaggcgcccggccagggtctcgaatggatgggggcaatctctggttctggtggttacactcactatgccgattcagtgaagggtcgcgtaactattaccgccgacgaatcaacctccaccgcctacatggaactcagctctctgaggtcagaagacacggccgtctattattgcgccagatctgcaactttcggtgtttgggaaactttcgatgtttggggtcagggcactttagtgaccgtctcatcg

SEQ ID NO: 227 - protein, 214 aa, Artificial Sequence
  Synthetic (23_LightChain_Kappa)
DIQMTQSPSSLSASVGDRVTITCRASQSISNYLNWYQQKPGKAPKLLIYDTSTLQSGVPSRFSGSGSGTDFTLTISSLQPEDFATYYCQQSYSFPWTFGQGTKVEIKRTVAAPSVFIFPPSDEQLKSGTASVVCLLNNFYPREAKVQWKVDNALQSGNSQESVTEQDSKDSTYSLSSTLTLSKADYEKHKVYACEVTHQGLSSPVTKSFNRGEC

SEQ ID NO: 228 - protein, 447 aa, Artificial Sequence
  Synthetic (23_HeavyChain)
QVQLVQSGAEVKKPGSSVKVSCKASGGTFSDYAMHWVRQAPGQGLEWMGAISGSGGYTHYADSVKGRVTITADESTSTAYMELSSLRSEDTAVYYCARSATFGVWETFDVWGQGTLVTVSSASTKGPSVFPLAPCSRSTSESTAALGCLVKDYFPEPVTVSWNSGALTSGVHTFPAVLQSSGLYSLSSVVTVPSSSLGTKTYTCNVDHKPSNTKVDKRVESKYGPPCPPCPAPEAAGGPSVFLFPPKPKDTLMISRTPEVTCVVVDVSQEDPEVQFNWYVDGVEVHNAKTKPREEQFNSTYRVVSVLTVLHQDWLNGKEYKCKVSNKGLPSSIEKTISKAKGQPREPQVYTLPPSQEEMTKNQVSLTCLVKGFYPSDIAVEWESNGQPENNYKTTPPVLDSDGSFFLYSRLTVDKSRWQEGNVFSCSVMHEALHNHYTQKSLSLSLG

SEQ ID NO: 229 - protein, 326 aa, Artificial Sequence
  Synthetic (IgG4_Fc)
ASTKGPSVFPLAPCSRSTSESTAALGCLVKDYFPEPVTVSWNSGALTSGVHTFPAVLQSSGLYSLSSVVTVPSSSLGTKTYTCNVDHKPSNTKVDKRVESKYGPPCPPCPAPEAAGGPSVFLFPPKPKDTLMISRTPEVTCVVVDVSQEDPEVQFNWYVDGVEVHNAKTKPREEQFNSTYRVVSVLTVLHQDWLNGKEYKCKVSNKGLPSSIEKTISKAKGQPREPQVYTLPPSQEEMTKNQVSLTCLVKGFYPSDIAVEWESNGQPENNYKTTPPVLDSDGSFFLYSRLTVDKSRWQEGNVFSCSVMHEALHNHYTQKSLSLSLG

SEQ ID NO: 230 - protein, 107 aa, Artificial Sequence [sequence omitted]